European Patent Application EP 4 678 651 A2, published January 14, 2026. Title: Branched peptides with antibacterial and anti-inflammatory activity. Applicant: Universita' degli Studi di Siena. Application EP. The sequence listing filed with the application follows.

SEQUENCE LISTING (21 sequences)

SEQ ID NO: 1 - protein, 12 aa, synthetic construct
TLLKKVLKAAAK

SEQ ID NO: 2 - protein, 11 aa, synthetic construct
LLKKVLLAAAK

SEQ ID NO: 3 - protein, 13 aa, synthetic construct
GIIDIAKKLFESW

SEQ ID NO: 4 - protein, 12 aa, synthetic construct
LRAAHRLAIGRR

SEQ ID NO: 5 - protein, 10 aa, synthetic construct
KLLKRIKKLL

SEQ ID NO: 6 - protein, 11 aa, synthetic construct
KKLLGKNWKLM

SEQ ID NO: 7 - protein, 10 aa, synthetic construct
LKKVLKAAAK

SEQ ID NO: 8 - protein, 9 aa, synthetic construct
LKLKSIVSW

SEQ ID NO: 9 - protein, 9 aa, synthetic construct
INLKKLAKL

SEQ ID NO: 10 - protein, 10 aa, synthetic construct
GRFKRFRKKL

SEQ ID NO: 11 - protein, 11 aa, synthetic construct
RGLRRLGRKIA

SEQ ID NO: 12 - protein, 12 aa, synthetic construct
  PEPTIDE 1..12: note = all AA are D-AA
TLLKKVLKAAAK

SEQ ID NO: 13 - protein, 14 aa, synthetic construct
INLKAIAALAKKLL

SEQ ID NO: 14 - protein, 12 aa, synthetic construct
LSAAHSLAIGRR

SEQ ID NO: 15 - protein, 12 aa, synthetic construct
LSAARSLAIGRR

SEQ ID NO: 16 - protein, 9 aa, synthetic construct
STVLTSKYR

SEQ ID NO: 17 - protein, 10 aa, synthetic construct
ALLKRIKTLL

SEQ ID NO: 18 - protein, 10 aa, synthetic construct
KLLKFIKTLL

SEQ ID NO: 19 - protein, 10 aa, synthetic construct
RGLRRLGRKI

SEQ ID NO: 20 - protein, 10 aa, synthetic construct
KRLWHKVGPF

SEQ ID NO: 21 - protein, 11 aa, synthetic construct
LLKKVLKAAAK